European Patent Specification EP 3 829 618 B1, published July 16, 2025. Title: Antigen Purification Method. Applicant: GSK Biologicals SA. The sequence listing filed with the application follows.

SEQUENCE LISTING (9 sequences)

SEQ ID NO: 1 - protein, 544 aa, RSV
MELLILKANAITTILTAVTFCFASGQNITEEFYQSTCSAVSKGYLSALRTGWYTSVITIELSNIKENKCNGTDAKVKLIKQELDKYKNAVTELQLLMQSTPATNNRARRELPRFMNYTLNNAKKTNVTLSKKRKRRFLGFLLGVGSAIASGVAVCKVLHLEGEVNKIKSALLSTNKAVVSLSNGVSVLTFKVLDLKNYIDKQLLPILNKQSCSISNIETVIEFQQKNNRLLEITREFSVNAGVTTPVSTYMLTNSELLSLINDMPITNDQKKLMSNNVQIVRQQSYSIMCIIKEEVLAYVVQLPLYGVIDTPCWKLHTSPLCTTNTKEGSNICLTRTDRGWYCDNAGSVSFFPQAETCKVQSNRVFCDTMNSLTLPSEVNLCNVDIFNPKYDCKIMTSKTDVSSSVITSLGAIVSCYGKTKCTASNKNRGIIKTFSNGCDYVSNKGVDTVSVGNTLYYVNKQEGKSLYVKGEPIINFYDPLVFPSDEFDASISQVNEKINQSLAFIRKSDELLSAIGGYIPEAPRDGQAYVRKDGEWVLLSTFL

SEQ ID NO: 2 - protein, 408 aa, RSV
FLGFLLGVGSAIASGVAVCKVLHLEGEVNKIKSALLSTNKAVVSLSNGVSVLTFKVLDLKNYIDKQLLPILNKQSCSISNIETVIEFQQKNNRLLEITREFSVNAGVTTPVSTYMLTNSELLSLINDMPITNDQKKLMSNNVQIVRQQSYSIMCIIKEEVLAYVVQLPLYGVIDTPCWKLHTSPLCTTNTKEGSNICLTRTDRGWYCDNAGSVSFFPQAETCKVQSNRVFCDTMNSLTLPSEVNLCNVDIFNPKYDCKIMTSKTDVSSSVITSLGAIVSCYGKTKCTASNKNRGIIKTFSNGCDYVSNKGVDTVSVGNTLYYVNKQEGKSLYVKGEPIINFYDPLVFPSDEFDASISQVNEKINQSLAFIRKSDELLSAIGGYIPEAPRDGQAYVRKDGEWVLLSTFL

SEQ ID NO: 3 - protein, 84 aa, RSV
QNITEEFYQSTCSAVSKGYLSALRTGWYTSVITIELSNIKENKCNGTDAKVKLIKQELDKYKNAVTELQLLMQSTPATNNRARR

SEQ ID NO: 4 - protein, 11 aa, RSV
KINQSLAFIRK

SEQ ID NO: 5 - protein, 11 aa, RSV
KIDQSLAFIRK

SEQ ID NO: 6 - protein, 10 aa, RSV
FMNYTLNNAK

SEQ ID NO: 7 - protein, 27 aa, RSV
ELPRFMNYTLNNAKKTNVTLSKKRKRR

SEQ ID NO: 8 - protein, 435 aa, RSV
ELPRFMNYTLNNAKKTNVTLSKKRKRRFLGFLLGVGSAIASGVAVCKVLHLEGEVNKIKSALLSTNKAVVSLSNGVSVLTFKVLDLKNYIDKQLLPILNKQSCSISNIETVIEFQQKNNRLLEITREFSVNAGVTTPVSTYMLTNSELLSLINDMPITNDQKKLMSNNVQIVRQQSYSIMCIIKEEVLAYVVQLPLYGVIDTPCWKLHTSPLCTTNTKEGSNICLTRTDRGWYCDNAGSVSFFPQAETCKVQSNRVFCDTMNSLTLPSEVNLCNVDIFNPKYDCKIMTSKTDVSSSVITSLGAIVSCYGKTKCTASNKNRGIIKTFSNGCDYVSNKGVDTVSVGNTLYYVNKQEGKSLYVKGEPIINFYDPLVFPSDEFDASISQVNEKINQSLAFIRKSDELLSAIGGYIPEAPRDGQAYVRKDGEWVLLSTFL

SEQ ID NO: 9 - protein, 5 aa, RSV
  misc_feature (2)..(2): Xaa can be any naturally occurring amino acid
  misc_feature (5)..(5): Xaa can be any naturally occurring amino acid
RXRRX